European Patent Application EP 4 299 743 A1, published January 3, 2024. Title: Nucleic acid medicine for expressing myostatin splicing variant. Applicant: Kobe Gakuin Educational Foundation. The sequence listing filed with the application follows.

SEQUENCE LISTING (70 sequences)

SEQ ID NO: 1 - DNA, 1939 bp, Homo sapiens
aatccgtttttagaggtcaaggtaacagacacaccaaaaagatccagaagggattttggtcttgactgtgatgagcactcaacagaatcacgatgctgtcgttaccctctaactgtggattttgaagcttttggatgggattggattatcgctcctaaaagatataaggccaattactgctctggagagtgtgaatttgtatttttacaaaaatatcctcatactcatctggtacaccaagcaaaccccagaggttcagcaggcccttgctgtactcccacaaagatgtctccaattaatatgctatattttaatggcaaagaacaaataatatatgggaaaattccagcgatggtagtagaccgctgtgggtgctcatgagatttatattaagcgttcataacttcctaaaacatggaaggttttcccctcaacaattttgaagctgtgaaattaagtaccacaggctataggcctagagtatgctacagtcacttaagcataagctacagtatgtaaactaaaagggggaatatatgcaatggttggcatttaaccatccaaacaaatcatacaagaaagttttatgatttccagagtttttgagctagaaggagatcaaattacatttatgttcctatatattacaacatcggcgaggaaatgaaagcgattctccttgagttctgatgaattaaaggagtatgctttaaagtctatttctttaaagttttgtttaatatttacagaaaaatccacatacagtattggtaaaatgcaggattgttatataccatcattcgaatcatccttaaacacttgaatttatattgtatggtagtatacttggtaagataaaattccacaaaaatagggatggtgcagcatatgcaatttccattcctattataattgacacagtacattaacaatccatgccaacggtgctaatacgataggctgaatgtctgaggctaccaggtttatcacataaaaaacattcagtaaaatagtaagtttctcttttcttcaggtgcattttcctacacctccaaatgaggaatggattttctttaatgtaagaagaatcatttttctagaggttggctttcaattctgtagcatacttggagaaactgcattatcttaaaaggcagtcaaatggtgtttgtttttatcaaaatgtcaaaataacatacttggagaagtatgtaattttgtctttggaaaattacaacactgcctttgcaacactgcagtttttatggtaaaataatagaaatgatcgactctatcaatattgtataaaaagactgaaacaatgcatttatataatatgtatacaatattgttttgtaaataagtgtctccttttttatttactttggtatatttttacactaaggacatttcaaattaagtactaaggcacaaagacatgtcatgcatcacagaaaagcaactacttatatttcagagcaaattagcagattaaatagtggtcttaaaactccatatgttaatgattagatggttatattacaatcattttatatttttttacatgattaacattcacttatggattcatgatggctgtataaagtgaatttgaaatttcaatggtttactgtcattgtgtttaaatctcaacgttccattattttaatacttgcaaaaacattactaagtataccaaaataattgactctattatctgaaatgaagaataaactgatgctatctcaacaataactgttacttttattttataatttgataatgaatatatttctgcatttatttacttctgttttgtaaattgggattttgttaatcaaatttattgtactatgactaaatgaaattatttcttacatctaatttgtagaaacagtataagttatattaaagtgttttcacatttttttgaaagaca

SEQ ID NO: 2 - DNA, 24 bp, Homo sapiens
ttagaggtcaaggtaacagacaca

SEQ ID NO: 3 - DNA, 18 bp, Artificial Sequence
  Antisense oligonucleotide
gaacaatcagtaatatca

SEQ ID NO: 4 - DNA, 18 bp, Artificial Sequence
  Antisense oligonucleotide
aaacggattctgtttgaa

SEQ ID NO: 5 - DNA, 18 bp, Artificial Sequence
  Antisense oligonucleotide
tcatcacagtcaagacca

SEQ ID NO: 6 - DNA, 18 bp, Artificial Sequence
  Antisense oligonucleotide
cctgctgaacctctgggg

SEQ ID NO: 7 - DNA, 18 bp, Artificial Sequence
  Antisense oligonucleotide
attgttgaggggaaaacc

SEQ ID NO: 8 - DNA, 18 bp, Artificial Sequence
  Antisense oligonucleotide
tatagcctgtggtactta

SEQ ID NO: 9 - DNA, 18 bp, Artificial Sequence
  Antisense oligonucleotide
cagtcaagaccaaaatcc

SEQ ID NO: 10 - DNA, 18 bp, Artificial Sequence
  Antisense oligonucleotide
cacagtcaagaccaaaat

SEQ ID NO: 11 - DNA, 18 bp, Artificial Sequence
  Antisense oligonucleotide
atcacagtcaagaccaaa

SEQ ID NO: 12 - DNA, 18 bp, Artificial Sequence
  Antisense oligonucleotide
gctcatcacagtcaagac

SEQ ID NO: 13 - DNA, 18 bp, Artificial Sequence
  Antisense oligonucleotide
gtgctcatcacagtcaag

SEQ ID NO: 14 - DNA, 18 bp, Artificial Sequence
  Antisense oligonucleotide
gagtgctcatcacagtca

SEQ ID NO: 15 - DNA, 18 bp, Artificial Sequence
  Antisense oligonucleotide
tccagagcagtaattggc

SEQ ID NO: 16 - DNA, 18 bp, Artificial Sequence
  Antisense oligonucleotide
tgagcacccacagcggtc

SEQ ID NO: 17 - DNA, 18 bp, Artificial Sequence
  Antisense oligonucleotide
ctcgccgatgttgtaata

SEQ ID NO: 18 - DNA, 18 bp, Artificial Sequence
  Antisense oligonucleotide
catatgctgcaccatccc

SEQ ID NO: 19 - DNA, 18 bp, Artificial Sequence
  Antisense oligonucleotide
tgtaggaaaatgcacctg

SEQ ID NO: 20 - DNA, 18 bp, Artificial Sequence
  Antisense oligonucleotide
caaaggcagtgttgtaat

SEQ ID NO: 21 - DNA, 18 bp, Artificial Sequence
  Antisense oligonucleotide
cccctaaggtcagtacca

SEQ ID NO: 22 - DNA, 18 bp, Artificial Sequence
  Antisense oligonucleotide
gttgaagtaataaactaa

SEQ ID NO: 23 - DNA, 18 bp, Artificial Sequence
  Antisense oligonucleotide
ggcctggaaacacttttc

SEQ ID NO: 24 - DNA, 18 bp, Artificial Sequence
  Antisense oligonucleotide
tgttaccttgacctctaa

SEQ ID NO: 25 - DNA, 18 bp, Artificial Sequence
  Antisense oligonucleotide
cttgacctctaaaaacgg

SEQ ID NO: 26 - DNA, 18 bp, Artificial Sequence
  Antisense oligonucleotide
taccttgacctctaaaaa

SEQ ID NO: 27 - DNA, 18 bp, Artificial Sequence
  Antisense oligonucleotide
gtctgttaccttgacctc

SEQ ID NO: 28 - DNA, 18 bp, Artificial Sequence
  Antisense oligonucleotide
tgtgtctgttaccttgac

SEQ ID NO: 29 - DNA, 18 bp, Artificial Sequence
  Antisense oligonucleotide
tggtgtgtctgttacctt

SEQ ID NO: 30 - DNA, 18 bp, Artificial Sequence
  Antisense oligonucleotide
ctgttaccttgacctcta

SEQ ID NO: 31 - DNA, 18 bp, Artificial Sequence
  Antisense oligonucleotide
tctgttaccttgacctct

SEQ ID NO: 32 - DNA, 18 bp, Artificial Sequence
  Antisense oligonucleotide
tgtctgttaccttgacct

SEQ ID NO: 33 - DNA, 18 bp, Artificial Sequence
  Antisense oligonucleotide
gtgtctgttaccttgacc

SEQ ID NO: 34 - DNA, 18 bp, Artificial Sequence
  Antisense oligonucleotide
gtgtgtctgttaccttga

SEQ ID NO: 35 - DNA, 18 bp, Artificial Sequence
  Antisense oligonucleotide
ggtgtgtctgttaccttg

SEQ ID NO: 36 - DNA, 18 bp, Artificial Sequence
  Antisense oligonucleotide
gcttcaaaatccacagtt

SEQ ID NO: 37 - DNA, 18 bp, Artificial Sequence
  Antisense oligonucleotide
tcttttaggagcgataat

SEQ ID NO: 38 - DNA, 18 bp, Artificial Sequence
  Antisense oligonucleotide
ggatatttttgtaaaaat

SEQ ID NO: 39 - DNA, 18 bp, Artificial Sequence
  Antisense oligonucleotide
agacatctttgtgggagt

SEQ ID NO: 40 - DNA, 18 bp, Artificial Sequence
  Antisense oligonucleotide
atatattatttgttcttt

SEQ ID NO: 41 - DNA, 18 bp, Artificial Sequence
  Antisense oligonucleotide
actctggaaatcataaaa

SEQ ID NO: 42 - DNA, 18 bp, Artificial Sequence
  Antisense oligonucleotide
taattcatcagaactcaa

SEQ ID NO: 43 - DNA, 18 bp, Artificial Sequence
  Antisense oligonucleotide
tgtaaatattaaacaaaa

SEQ ID NO: 44 - DNA, 18 bp, Artificial Sequence
  Antisense oligonucleotide
cagcctatcgtattagca

SEQ ID NO: 45 - DNA, 18 bp, Artificial Sequence
  Antisense oligonucleotide
ctggtagcctcagacatt

SEQ ID NO: 46 - DNA, 18 bp, Artificial Sequence
  Antisense oligonucleotide
ccgttggcatggattgtt

SEQ ID NO: 47 - DNA, 18 bp, Artificial Sequence
  Antisense oligonucleotide
gttttttatgtgataaac

SEQ ID NO: 48 - DNA, 18 bp, Artificial Sequence
  Antisense oligonucleotide
agagaaacttactatttt

SEQ ID NO: 49 - DNA, 18 bp, Artificial Sequence
  Antisense oligonucleotide
tcttacattaaagaaaat

SEQ ID NO: 50 - DNA, 18 bp, Artificial Sequence
  Antisense oligonucleotide
tgaaagccaacctctaga

SEQ ID NO: 51 - DNA, 18 bp, Artificial Sequence
  Antisense oligonucleotide
ataaaaacaaacaccatt

SEQ ID NO: 52 - DNA, 18 bp, Artificial Sequence
  Antisense oligonucleotide
tttctattattttaccat

SEQ ID NO: 53 - DNA, 18 bp, Artificial Sequence
  Antisense oligonucleotide
aaagtaaataaaaaagga

SEQ ID NO: 54 - DNA, 18 bp, Artificial Sequence
  Antisense oligonucleotide
tgtccttagtgtaaaaat

SEQ ID NO: 55 - DNA, 18 bp, Artificial Sequence
  Antisense oligonucleotide
ttctgtgatgcatgacat

SEQ ID NO: 56 - DNA, 18 bp, Artificial Sequence
  Antisense oligonucleotide
tcatgtaaaaaaatataa

SEQ ID NO: 57 - DNA, 20 bp, Artificial Sequence
  Primer
agattcactggtgtggcaag

SEQ ID NO: 58 - DNA, 20 bp, Artificial Sequence
  Primer
tgcatgacatgtctttgtgc

SEQ ID NO: 59 - DNA, 18 bp, Artificial Sequence
  Primer
cccttcattgacctcaac

SEQ ID NO: 60 - DNA, 18 bp, Artificial Sequence
  Primer
ttcacacccatgacgaac

SEQ ID NO: 61 - DNA, 18 bp, Artificial Sequence
  Antisense oligonucleotide
tctgutaccutgacctct

SEQ ID NO: 62 - DNA, 18 bp, Artificial Sequence
  Antisense oligonucleotide
tctgutaccttgacctct

SEQ ID NO: 63 - DNA, 18 bp, Artificial Sequence
  Antisense oligonucleotide
tctguuacctugacctct

SEQ ID NO: 64 - DNA, 18 bp, Artificial Sequence
  Antisense oligonucleotide
tctgutacctugacctct

SEQ ID NO: 65 - DNA, 18 bp, Artificial Sequence
  Antisense oligonucleotide
tctgutacctugaccuct

SEQ ID NO: 66 - DNA, 18 bp, Artificial Sequence
  Antisense oligonucleotide
tctguuaccutgacctct

SEQ ID NO: 67 - DNA, 18 bp, Artificial Sequence
  Antisense oligonucleotide
tctguuaccutgaccuct

SEQ ID NO: 68 - DNA, 1860 bp, Homo sapiens
agattcactggtgtggcaagttgtctctcagactgtacatgcattaaaattttgcttggcattactcaaaagcaaaagaaaagtaaaaggaagaaacaagaacaagaaaaaagattatattgattttaaaatcatgcaaaaactgcaactctgtgtttatatttacctgtttatgctgattgttgctggtccagtggatctaaatgagaacagtgagcaaaaagaaaatgtggaaaaagaggggctgtgtaatgcatgtacttggagacaaaacactaaatcttcaagaatagaagccattaagatacaaatcctcagtaaacttcgtctggaaacagctcctaacatcagcaaagatgttataagacaacttttacccaaagctcctccactccgggaactgattgatcagtatgatgtccagagggatgacagcagcgatggctctttggaagatgacgattatcacgctacaacggaaacaatcattaccatgcctacagagtctgattttctaatgcaagtggatggaaaacccaaatgttgcttctttaaatttagctctaaaatacaatacaataaagtagtaaaggcccaactatggatatatttgagacccgtcgagactcctacaacagtgtttgtgcaaatcctgagactcatcaaacctatgaaagacggtacaaggtatactggaatccgatctctgaaacttgacatgaacccaggcactggtatttggcagagcattgatgtgaagacagtgttgcaaaattggctcaaacaacctgaatccaacttaggcattgaaataaaagctttagatgagaatggtcatgatcttgctgtaaccttcccaggaccaggagaagatgggctgaatgtctgaggctaccaggtttatcacataaaaaacattcagtaaaatagtaagtttctcttttcttcaggtgcattttcctacacctccaaatgaggaatggattttctttaatgtaagaagaatcatttttctagaggttggctttcaattctgtagcatacttggagaaactgcattatcttaaaaggcagtcaaatggtgtttgtttttatcaaaatgtcaaaataacatacttggagaagtatgtaattttgtctttggaaaattacaacactgcctttgcaacactgcagtttttatggtaaaataatagaaatgatcgactctatcaatattgtataaaaagactgaaacaatgcatttatataatatgtatacaatattgttttgtaaataagtgtctccttttttatttactttggtatatttttacactaaggacatttcaaattaagtactaaggcacaaagacatgtcatgcatcacagaaaagcaactacttatatttcagagcaaattagcagattaaatagtggtcttaaaactccatatgttaatgattagatggttatattacaatcattttatatttttttacatgattaacattcacttatggattcatgatggctgtataaagtgaatttgaaatttcaatggtttactgtcattgtgtttaaatctcaacgttccattattttaatacttgcaaaaacattactaagtataccaaaataattgactctattatctgaaatgaagaataaactgatgctatctcaacaataactgttacttttattttataatttgataatgaatatatttctgcatttatttacttctgttttgtaaattgggattttgttaatcaaatttattgtactatgactaaatgaaattatttcttacatctaatttgtagaaacagtataagttatattaaagtgttttcacatttttttgaaagacaaaaa

SEQ ID NO: 69 - protein, 251 aa, Homo sapiens [sequence omitted]

SEQ ID NO: 70 - protein, 375 aa, Homo sapiens
MQKLQLCVYIYLFMLIVAGPVDLNENSEQKENVEKEGLCNACTWRQNTKSSRIEAIKIQILSKLRLETAPNISKDVIRQLLPKAPPLRELIDQYDVQRDDSSDGSLEDDDYHATTETIITMPTESDFLMQVDGKPKCCFFKFSSKIQYNKVVKAQLWIYLRPVETPTTVFVQILRLIKPMKDGTRYTGIRSLKLDMNPGTGIWQSIDVKTVLQNWLKQPESNLGIEIKALDENGHDLAVTFPGPGEDGLNPFLEVKVTDTPKRSRRDFGLDCDEHSTESRCCRYPLTVDFEAFGWDWIIAPKRYKANYCSGECEFVFLQKYPHTHLVHQANPRGSAGPCCTPTKMSPINMLYFNGKEQIIYGKIPAMVVDRCGCS